European Patent Application EP 4 209 589 A1, published July 12, 2023. Title: Complex for modifying double-stranded DNA containing miniaturized cytidine deaminase. Applicant: NATIONAL UNIVERSITY CORPORATION KOBE UNIVERSITY. The sequence listing filed with the application follows.

SEQUENCE LISTING (24 sequences)

SEQ ID NO: 1 - protein, 208 aa, Petromyzon marinus
MTDAEYVRIHEKLDIYTFKKQFFNNKKSVSHRCYVLFELKRRGERRACFWGYAVNKPQSGTERGIHAEIFSIRKVEEYLRDNPGQFTINWYSSWSPCADCAEKILEWYNQELRGNGHTLKIWACKLYYEKNARNQIGLWNLRDNGVGLNVMVSEHYQCCRKIFIQSSHNQLNENRWLEKTLKRAEKRRSELSIMIQVKILHTTKSPAV

SEQ ID NO: 2 - protein, 121 aa, Petromyzon marinus
SHRCYVLFELKRRGERRACFWGYAVNKPQSGTERGIHAEIFSIRKVEEYLRDNPGQFTINWYSSWSPCADCAEKILEWYNQELRGNGHTLKIEACKLYYEKNARNQIGLQNLRDNGVGLNV

SEQ ID NO: 3 - protein, 198 aa, Homo sapiens [sequence omitted]

SEQ ID NO: 4 - protein, 1368 aa, Streptococcus pyogenes
MDKKYSIGLDIGTNSVGWAVITDDYKVPSKKFKVLGNTDRHSIKKNLIGALLFDSGEIAEATRLKRTARRRYTRRKNRICYLQEIFSNEMAKVDDSFFHRLEESFLVEEDKKHERHPIFGNIVDEVAYHEKYPTIYHLRKKLVDSTDKADLRLIYLALAHMIKFRGHFLIEGDLNPDNSDVDKLFIQLVQTYNQLFEENPINASGVDAKAILSARLSKSRRLENLIAQLPGEKKNGLFGNLIALSLGLTPNFKSNFDLAEDAKLQLSKDTYDDDLDNLLAQIGDQYADLFLAAKNLSDAILLSDILRLNSEITKAPLSASMIKRYDEHHQDLTLLKALVRQQLPEKYKEIFFDQSKNGYAGYIDGGASQEEFYKFIKPILEKMDGTEELLAKLNRKDLLRKQRTFDNGSIPHQIHLGELHAILRRQEDFYPFLKDNREKIEKILTFRIPYYVGPLARGNSRFAWMTRKSEETITPWNFEEVVDKGASAQSFIERMTNFDKNLPNEKVLPKHSLLYEYFTVYNELTKVKYVTEGMRKPAFLSGEQKKAIVDLLFKTNRKVTVKQLKEDYFKKIECFDSVEISGVEDRFNASLGTYHDLLKIIKDKDFLDNEENEDILEDIVLTLTLFEDREMIEERLKTYAHLFDDKVMKQLKRRRYTGWGRLSRKLINGIRDKQSGKTILDFLKSDGFANRNFMQLIHDDSLTFKEDIQKAQVSGQGDSLHEHIANLAGSPAIKKGILQTVKVVDELVKVMGRHKPENIVIEMARENQTTQKGQKNSRERMKRIEEGIKELGSQILKEHPVENTQLQNEKLYLYYLQNGRDMYVDQELDINRLSDYDVDHIVPQSFIKDDSIDNKVLTRSDKNRGKSDNVPSEEVVKKMKNYWRQLLNAKLITQRKFDNLTKAERGGLSELDKAGFIKRQLVETRQITKHVAQILDSRMNTKYDENDKLIREVKVITLKSKLVSDFRKDFQFYKVREINNYHHAHDAYLNAVVGTALIKKYPKLESEFVYGDYKVYDVRKMLAKSEQEIGKATAKYFFYSNIMNFFKTEITLANGEIRKRPLIETNGETGEIVWDKGRDFATVRKVLSMPQVNIVKKTEVQTGGFSKESILPKRNSDKLIARKKDWDPKKYGGFDSPTVAYSVLVVAKVEKGKSKKLKSVKELLGITIMERSSFEKNPIDFLEAKGYKEVRKDLIIKLPKYSLFELENGRKRMLASAGELQKGNELALPSKYVNFLYLASHYEKLKGSPEDNEQKQLFVEQHKHYLDEIIEQISEFSKRVILADANLDKVLSAYNKHRDKPIREQAENIIHLFTLTNLGAPTAFKYFDTTIDRKRYTSTKEVLDATFIHQSITGLYETRIDLSQLGGD

SEQ ID NO: 5 - protein, 1053 aa, Staphylococcus aureus
MKRNYILGLDIGITSVGYGIIDYETRDVIDAGVRLFKEANVENNEGRRSKRGARRLKRRRRHRIQRVKKLLFDYNLLTDHSELSGINPYEARVKGLSQKLSEEEFSAALLHLAKRRGVHNVNEVEEDTGNELSTKEQISRNSKALEEKYVAELQLERLKKDGEVRGSINRFKTSDYVKEAKQLLKVQKAYHQLDQSFIDTYIDLLETRRTYYEGPGEGSPFGWKDIKEWYEMLMGHCTYFPEELRSVKYAYNADLYNALNDLNNLVITRDENEKLEYYEKFQIIENVFKQKKKPTLKQIAKEILVNEEDIKGYRVTSTGKPEFTNLKVYHDIKDITARKEIIENAELLDQIAKILTIYQSSEDIQEELTNLNSELTQEEIEQISNLKGYTGTHNLSLKAINLILDELWHTNDNQIAIFNRLKLVPKKVDLSQQKEIPTTLVDDFILSPVVKRSFIQSIKVINAIIKKYGLPNDIIIELAREKNSKDAQKMINEMQKRNRQTNERIEEIIRTTGKENAKYLIEKIKLHDMQEGKCLYSLEAIPLEDLLNNPFNYEVDHIIPRSVSFDNSFNNKVLVKQEENSKKGNRTPFQYLSSSDSKISYETFKKHILNLAKGKGRISKTKKEYLLEERDINRFSVQKDFINRNLVDTRYATRGLMNLLRSYFRVNNLDVKVKSINGGFTSFLRRKWKFKKERNKGYKHHAEDALIIANADFIFKEWKKLDKAKKVMENQMFEEKQAESMPEIETEQEYKEIFITPHQIKHIKDFKDYKYSHRVDKKPNRELINDTLYSTRKDDKGNTLIVNNLNGLYDKDNDKLKKLINKSPEKLLMYHHDPQTYQKLKLIMEQYGDEKNPLYKYYEETGNYLTKYSKKDNGPVIKKIKYYGNKLNAHLDITDDYPNSRNKVVKLSLKPYRFDVYLDNGVYKFVTVKNLDVIKKENYYEVNSKCYEEAKKLKKISNQAEFIASFYNNDLIKINGELYRVIGVNNDLLNRIEVNMIDITYREYLENMNDKRPPRIIKTIASKTQSIKKYSTDILGNLYEVKSKKHPQIIKKG

SEQ ID NO: 6 - DNA, 83 bp, Streptococcus pyogenes
gttttagagctagaaatagcaagttaaaataaggctagtccgttatcaacttgaaaaagtggcaccgagtcggtgcttttttt

SEQ ID NO: 7 - DNA, 83 bp, Staphylococcus aureus
gttttagtactctggaaacagaatctactaaaacaaggcaaaatgccgtgtttatctcgtcaacttgttggcgagattttttt

SEQ ID NO: 8 - DNA, 20 bp, Artificial Sequence
  target sequence of gRNA (vector 1086)
gcccagttggattccgttat

SEQ ID NO: 9 - DNA, 20 bp, Artificial Sequence
  target sequence of gRNA (vector 1150)
ctccaataacggaatccaac

SEQ ID NO: 10 - DNA, 20 bp, Artificial Sequence
  target sequence of gRNA (vector 1025)
gatacgttctctatggagga

SEQ ID NO: 11 - DNA, 20 bp, Artificial Sequence
  target sequence of gRNA (vector 1149)
tccaataacggaatccaact

SEQ ID NO: 12 - DNA, 11741 bp, Artificial Sequence
  full-length sequence of vector pAL008
  rep_origin (70)..(573): CEN/ARS
  promoter (610)..(714): AmpR promoter
  gene (715)..(1575): AmpR
  rep_origin (1746)..(2334): ori
  promoter (2658)..(2688): lac promoter
  misc_feature (2696)..(2712)
  promoter (2853)..(3517): GAL1,10 promoter
  gene (3527)..(4150): PmCDA1
  mutation (3950)..(3955): H130A R131E
  mutation (3992)..(3994): Y146E for solubility
  mutation (4010)..(4150): truncated 161
  mutation (4055)..(4150): truncated 176
  gene (4163)..(8254): Cas9(D10A)
  sig_peptide (8267)..(8287): SV40 NLS
  terminator (8321)..(8508): ADH1 terminator
  rep_origin (8813)..(9268): f1 ori
  promoter (9568)..(9972): LEU2 promoter
  gene (9985)..(11079): LEU2
gacgaaagggcctcgtgatacgcctatttttataggttaatgtcatgataataatggtttcttaggacggatcgcttgcctgtaacttacacgcgcctcgtatcttttaatgatggaataatttgggaatttactctgtgtttatttatttttatgttttgtatttggattttagaaagtaaataaagaaggtagaagagttacggaatgaagaaaaaaaaataaacaaaggtttaaaaaatttcaacaaaaagcgtactttacatatatatttattagacaagaaaagcagattaaatagatatacattcgattaacgataagtaaaatgtaaaatcacaggattttcgtgtgtggtcttctacacagacaagatgaaacaattcggcattaatacctgagagcaggaagagcaagataaaaggtagtatttgttggcgatccccctagagtcttttacatcttcggaaaacaaaaactattttttctttaatttctttttttactttctatttttaatttatatatttatattaaaaaatttaaattataattatttttatagcacgtgatgaaaaggacccaggtggcacttttcggggaaatgtgcgcggaacccctatttgtttatttttctaaatacattcaaatatgtatccgctcatgagacaataaccctgataaatgcttcaataatattgaaaaaggaagagtatgagtattcaacatttccgtgtcgcccttattcccttttttgcggcattttgccttcctgtttttgctcacccagaaacgctggtgaaagtaaaagatgctgaagatcagttgggtgcacgagtgggttacatcgaactggatctcaacagcggtaagatccttgagagttttcgccccgaagaacgttttccaatgatgagcacttttaaagttctgctatgtggcgcggtattatcccgtattgacgccgggcaagagcaactcggtcgccgcatacactattctcagaatgacttggttgagtactcaccagtcacagaaaagcatcttacggatggcatgacagtaagagaattatgcagtgctgccataaccatgagtgataacactgcggccaacttacttctgacaacgatcggaggaccgaaggagctaaccgctttttttcacaacatgggggatcatgtaactcgccttgatcgttgggaaccggagctgaatgaagccataccaaacgacgagcgtgacaccacgatgcctgtagcaatggcaacaacgttgcgcaaactattaactggcgaactacttactctagcttcccggcaacaattaatagactggatggaggcggataaagttgcaggaccacttctgcgctcggcccttccggctggctggtttattgctgataaatctggagccggtgagcgtgggtctcgcggtatcattgcagcactggggccagatggtaagccctcccgtatcgtagttatctacacgacgggcagtcaggcaactatggatgaacgaaatagacagatcgctgagataggtgcctcactgattaagcattggtaactgtcagaccaagtttactcatatatactttagattgatttaaaacttcatttttaatttaaaaggatctaggtgaagatcctttttgataatctcatgaccaaaatcccttaacgtgagttttcgttccactgagcgtcagaccccgtagaaaagatcaaaggatcttcttgagatcctttttttctgcgcgtaatctgctgcttgcaaacaaaaaaaccaccgctaccagcggtggtttgtttgccggatcaagagctaccaactctttttccgaaggtaactggcttcagcagagcgcagataccaaatactgtccttctagtgtagccgtagttaggccaccacttcaagaactctgtagcaccgcctacatacctcgctctgctaatcctgttaccagtggctgctgccagtggcgataagtcgtgtcttaccgggttggactcaagacgatagttaccggataaggcgcagcggtcgggctgaacggggggttcgtgcacacagcccagcttggagcgaacgacctacaccgaactgagatacctacagcgtgagcattgagaaagcgccacgcttcccgaagggagaaaggcggacaggtatccggtaagcggcagggtcggaacaggagagcgcacgagggagcttccaggggggaacgcctggtatctttatagtcctgtcgggtttcgccacctctgacttgagcgtcgatttttgtgatgctcgtcaggggggccgagcctatggaaaaacgccagcaacgcggcctttttacggttcctggccttttgctggccttttgctcacatgttctttcctgcgttatcccctgattctgtggataaccgtattaccgcctttgagtgagctgataccgctcgccgcagccgaacgaccgagcgcagcgagtcagtgagcgaggaagcggaagagcgcccaatacgcaaaccgcctctccccgcgcgttggccgattcattaatgcagctggcacgacaggtttcccgactggaaagcgggcagtgagcgcaacgcaattaatgtgagttacctcactcattaggcaccccaggctttacactttatgcttccggctcctatgttgtgtggaattgtgagcggataacaatttcacacaggaaacagctatgaccatgattacgccaagctcggaattaaccctcactaaagggaacaaaagctgggtaccgggcccgaattctctccttctcttaggtggcagagcaggtggagggtcgaccatactagtttcaaaaattcttactttttttttggatggacgcaaagaagtttaataatcatattacatggcattaccaccatatacatatccatatacatatccatatctaatcttacttatatgttgtggaaatgtaaagagccccattatcttagcctaaaaaaaccttctctttggaactttcagtaatacgcttaactgctcattgctatattgaagtacggattagaagccgccgagcgggtgacagccctccgaaggaagactctcctccgtgcgtcctcgtcttcaccggtcgcgttcctgaaacgcagatgtgcctcgcgccgcactgctccgaacaataaagattctacaatactagcttttatggttatgaagaggaaaaattggcagtaacctggccccacaaaccttcaaatgaacgaatcaaattaacaaccataggatgataatgcgattagttttttagccttatttctggggtaattaatcagcgaagcgatgatttttgatctattaacagatatataaatgcaaaaactgcataaccactttaactaatactttcaacattttcggtttgtattacttcttattcaaatgtaataaaagtatcaacaaaaaattgttaatatacctctatactttaacgtcaaggagaaaaaaccgctcttcgatgaccgacgctgagtacgtgagaatccatgagaagttggacatctacacgtttaagaaacagtttttcaacaacaaaaaatccgtgtcgcatagatgctacgttctctttgaattaaaacgacggggtgaacgtagagcgtgtttttggggctatgctgtgaataaaccacagagcgggacagaacgtggcattcacgccgaaatctttagcattagaaaagtcgaagaatacctgcgcgacaaccccggacaattcacgataaattggtactcatcctggagtccttgtgcagattgcgctgaaaagatcttagaatggtataaccaggagctgcgggggaacggccacactttgaaaatctgggcttgcaaactctattacgagaaaaatgcgaggaatcaaattgggctgtggaacctcagagataacggggttgggttgaatgtaatggtaagtgaacactaccaatgttgcaggaaaatattcatccaatcgtcgcacaatcaattgaatgagaatagatggcttgagaagactttgaagcgagctgaaaaacgacggagcgagttgtccattatgattcaggtaaaaatactccacaccactaagagtcctgctgttatggacaagaagtactccattgggctcgctatcggcacaaacagcgtcggttgggccgtcattacggacgagtacaaggtgccgagcaaaaaattcaaagttctgggcaataccgatcgccacagcataaagaagaacctcattggcgccctcctgttcgactccggggagacggccgaagccacgcggctcaaaagaacagcacggcgcagatatacccgcagaaagaatcggatctgctacctgcaggagatctttagtaatgagatggctaaggtggatgactctttcttccataggctggaggagtcctttttggtggaggaggataaaaagcacgagcgccacccaatctttggcaatatcgtggacgaggtggcgtaccatgaaaagtacccaaccatatatcatctgaggaagaagcttgtagacagtactgataaggctgacttgcggttgatctatctcgcgctggcgcatatgatcaaatttcggggacacttcctcatcgagggggacctgaacccagacaacagcgatgtcgacaaactctttatccaactggttcagacttacaatcagcttttcgaagagaacccgatcaacgcatccggagttgacgccaaagcaatcctgagcgctaggctgtccaaatcccggcggctcgaaaacctcatcgcacagctccctggggagaagaagaacggcctgtttggtaatcttatcgccctgtcactcgggctgacccccaactttaaatctaacttcgacctggccgaagatgccaagcttcaactgagcaaagacacctacgatgatgatctcgacaatctgctggcccagatcggcgaccagtacgcagacctttttttggcggcaaagaacctgtcagacgccattctgctgagtgatattctgcgagtgaacacggagatcaccaaagctccgctgagcgctagtatgatcaagcgctatgatgagcaccaccaagacttgactttgctgaaggcccttgtcagacagcaactgcctgagaagtacaaggaaattttcttcgatcagtctaaaaatggctacgccggatacattgacggcggagcaagccaggaggaattttacaaatttattaagcccatcttggaaaaaatggacggcaccgaggagctgctggtaaagcttaacagagaagatctgttgcgcaaacagcgcactttcgacaatggaagcatcccccaccagattcacctgggcgaactgcacgctatcctcaggcggcaagaggatttctacccctttttgaaagataacagggaaaagattgagaaaatcctcacatttcggataccctactatgtaggccccctcgcccggggaaattccagattcgcgtggatgactcgcaaatcagaagagaccatcactccctggaacttcgaggaagtcgtggataagggggcctctgcccagtccttcatcgaaaggatgactaactttgataaaaatctgcctaacgaaaaggtgcttcctaaacactctctgctgtacgagtacttcacagtttataacgagctcaccaaggtcaaatacgtcacagaagggatgagaaagccagcattcctgtctggagagcagaagaaagctatcgtggacctcctcttcaagacgaaccggaaagttaccgtgaaacagctcaaagaagactatttcaaaaagattgaatgtttcgactctgttgaaatcagcggagtggaggatcgcttcaacgcatccctgggaacgtatcacgatctcctgaaaatcattaaagacaaggacttcctggacaatgaggagaacgaggacattcttgaggacattgtcctcacccttacgttgtttgaagatagggagatgattgaagaacgcttgaaaacttacgctcatctcttcgacgacaaagtcatgaaacagctcaagaggcgccgatatacaggatgggggcggctgtcaagaaaactgatcaatgggatccgagacaagcagagtggaaagacaatcctggattttcttaagtccgatggatttgccaaccggaacttcatgcagttgatccatgatgactctctcacctttaaggaggacatccagaaagcacaagtttctggccagggggacagtcttcacgagcacatcgctaatcttgcaggtagcccagctatcaaaaagggaatactgcagaccgttaaggtcgtggatgaactcgtcaaagtaatgggaaggcataagcccgagaatatcgttatcgagatggcccgagagaaccaaactacccagaagggacagaagaacagtagggaaaggatgaagaggattgaagagggtataaaagaactggggtcccaaatccttaaggaacacccagttgaaaacacccagcttcagaatgagaagctctacctgtactacctgcagaacggcagggacatgtacgtggatcaggaactggacatcaatcggctctccgactacgacgtggatcatatcgtgccccagtcttttctcaaagatgattctattgataataaagtgttgacaagatccgataaaaatagagggaagagtgataacgtcccctcagaagaagttgtcaagaaaatgaaaaattattggcggcagctgctgaacgccaaactgatcacacaacggaagttcgataatctgactaaggctgaacgaggtggcctgtctgagttggataaagccggcttcatcaaaaggcagcttgttgagacacgccagatcaccaagcacgtggcccaaattctcgattcacgcatgaacaccaagtacgatgaaaatgacaaactgattcgagaggtgaaagttattactctgaagtctaagctggtctcagatttcagaaaggactttcagttttataaggtgagagagatcaacaattaccaccatgcgcatgatgcctacctgaatgcagtggtaggcactgcacttatcaaaaaatatcccaagcttgaatctgaatttgtttacggagactataaagtgtacgatgttaggaaaatgatcgcaaagtctgagcaggaaataggcaaggccaccgctaagtacttcttttacagcaatattatgaattttttcaagaccgagattacactggccaatggagagattcggaagcgaccacttatcgaaacaaacggagaaacaggagaaatcgtgtgggacaagggtagggatttcgcgacagtccggaaggtcctgtccatgccgcaggtgaacatcgttaaaaagaccgaagtacagaccggaggcttctccaaggaaagtatcctcccgaaaaggaacagcgacaagctgatcgcacgcaaaaaagattgggaccccaagaaatacggcggattcgattctcctacagtcgcttacagtgtactggttgtggccaaagtggagaaagggaagtctaaaaaactcaaaagcgtcaaggaactgctgggcatcacaatcatggagcgatcaagcttcgaaaaaaaccccatcgactttctcgaggcgaaaggatataaagaggtcaaaaaagacctcatcattaagcttcccaagtactctctctttgagcttgaaaacggccggaaacgaatgctcgctagtgcgggcgagctgcagaaaggtaacgagctggcactgccctctaaatacgttaatttcttgtatctggccagccactatgaaaagctcaaagggtctcccgaagataatgagcagaagcagctgttcgtggaacaacacaaacactaccttgatgagatcatcgagcaaataagcgaattctccaaaagagtgatcctcgccgacgctaacctcgataaggtgctttctgcttacaataagcacagggataagcccatcagggagcaggcagaaaacattatccacttgtttactctgaccaacttgggcgcgcctgcagccttcaagtacttcgacaccaccatagacagaaagcggtacacctctacaaaggaggtcctggacgccacactgattcatcagtcaattacggggctctatgaaacaagaatcgacctctctcagctcggtggagacagcagggctgaccccaagaagaagaggaaggtgtagtctagaggctccggataaggatcctaataagcgaatttcttatgatttatgatttttattattaaataagttataaaaaaaataagtgtatacaaattttaaagtgactcttaggttttaaaacgaaaattcttattcttgagtaactctttcctgtaggtcaggttgctttctcaggtatagcatgaggtcgctcttattgaccacacctctaccggcatgccgagcaaatgcctgcaaatcgctcccgggcaaaaaaccccctcaagacccgtttagaggccccaaggggttatgctatgcataccaagcttccgcggtggagctccaattcgccctatagtgagtcgtattacaattcactggccgtcgttttacaacgtcgtgactgggaaaaccctggcgttacccaacttaatcgccttgcagcacatccccccttcgccagctggcgtaatagcgaagaggcccgcaccgatcgcccttcccaacagttgcgcagcctgaatggcgaatggcgcgacgcgccctgtagcggcgcattaagcgcggcgggtgtggtggttacgcgcagcgtgaccgctacacttgccagcgccctagcgcccgctcctttcgctttcttcccttcctttctcgccacgttcgccggctttccccgtcaagctctaaatcgggggctccctttagggttccgatttagtgctttacggcacctcgaccccaaaaaacttgattagggtgatggttcacgtagtgggccatcgccctgatagacggtttttcgccctttgacgttggagtccacgttctttaatagtggactcttgttccaaactggaacaacactcaaccctatctcggtctattcttttgatttataagggattttgccgatttcggcctattggttaaaaaatgagctgatttaacaaaaatttaacgcgaattttaacaaaatattaacgtttacaatttcctgatgcggtattttctccttacgcatctgtgcggtatttcacaccgcatatcgaccctcgaggagaacttctagtatatccacatacctaatattattgccttattaaaaatggaatcggaacaattacatcaaaatccacattctcttcaaaatcaattgtcctgtacttccttgttcatgtgtgttcaaaaacgttatatttataggataattatactctatttctcaacaagtaattggttgtttggccgagcggtctaaggcgcctgattcaagaaatatcttgaccgcagttaactgtgggaatactcaggtatcgtaagatgcaagagttcgaatctcttagcaaccattatttttttcctcaacataacgagaacacacaggggcgctatcgcacagaatcaaattcgatgactggaaattttttgttaatttcagaggtcgcctgacgcatatacctttttcaactgaaaaattgggagaaaaaggaaaggtgagaggccggaaccggcttttcatatagaatagagaagcgttcatgactaaatgcttgcatcacaatacttgaagttgacaatattatttaaggacctattgttttttccaataggtggttagcaatcgtcttactttctaacttttcttaccttttacatttcagcaatatatatatatatttcaaggatataccattctaatgtctgcccctatgtctgcccctaagaagatcgtcgttttgccaggtgaccacgttggtcaagaaatcacagccgaagccattaaggttcttaaagctatttctgatgttcgttccaatgtcaagttcgatttcgaaaatcatttaattggtggtgctgctatcgatgctacaggtgtcccacttccagatgaggcgctggaagcctccaagaaggttgatgccgttttgttaggtgctgtgggtggtcctaaatggggtaccggtagtgttagacctgaacaaggtttactaaaaatccgtaaagaacttcaattgtacgccaacttaagaccatgtaactttgcatccgactctcttttagacttatctccaatcaagccacaatttgctaaaggtactgacttcgttgttgtcagagaattagtgggaggtatttactttggtaagagaaaggaagacgatggtgatggtgtcgcttgggatagtgaacaatacaccgttccagaagtgcaaagaatcacaagaatggccgctttcatggccctacaacatgagccaccattgcctatttggtccttggataaagctaatgttttggcctcttcaagattatggagaaaaactgtggaggaaaccatcaagaacgaattccctacattgaaggttcaacatcaattgattgattctgccgccatgatcctagttaagaacccaacccacctaaatggtattataatcaccagcaacatgtttggtgatatcatctccgatgaagcctccgttatcccaggttccttgggtttgttgccatctgcgtccttggcctctttgccagacaagaacaccgcatttggtttgtacgaaccatgccacggttctgctccagatttgccaaagaataaggttgaccctatcgccactatcttgtctgctgcaatgatgttgaaattgtcattgaacttgcctgaagaaggtaaggccattgaagatgcagttaaaaaggttttggatgcaggtatcagaactggtgatttaggtggttccaacagtaccaccgaagtcggtgatgctgtcgccgaagaagttaagaaaatccttgcttaaaaagattctctttttttatgatatttgtacataaactttataaatgaaattcataatagaaacgacacgaaattacaaaatggaatatgttcatagggtagacgaaactatatacgcaatctacatacatttatcaagaaggagaaaaaggaggatagtaaaggaatacaggtaagcaaattgatactaatggctcaacgtgataaggaaaaagaattgcactttaacattaatattgacaaggaggagggcaccacacaaaaagttaggtgtaacagaaaatcatgaaactacgattcctaatttgatattggaggattttctctaaaaaaaaaaaaatacaacaaataaaaaacactcaatgacctgaccatttgatggagtttaagtcaataccttcttgaaccatttcccataatggtgaaagttccctcaagaattttactctgtcagaaacggccttacgacgtagtcgatatggtgcactctcagtacaatctgctctgatgccgcatagttaagccagccccgacacccgccaacacccgctgacgcgccctgacgggcttgtctgctcccggcatccgcttacagacaagctgtgaccgtctccgggagctgcatgtgtcagaggttttcaccgtcatcaccgaaacgcgcga

SEQ ID NO: 13 - DNA, 11575 bp, Artificial Sequence
  full-length sequence of vector pAL022
  rep_origin (70)..(573): CEN/ARS
  promoter (610)..(714): AmpR promoter
  gene (715)..(1575): AmpR
  rep_origin (1746)..(2334): ori
  promoter (2658)..(2688): lac promoter
  misc_feature (2696)..(2712): lac operator
  promoter (2852)..(3516): GAL1,10 promoter
  misc_feature (3068)..(3185): UAS
  gene (3532)..(3894): PmCDA1
  mutation (3820)..(3822): Expsose N (V150 Y128 interaction)
  mutation (3826)..(3828): Expose Q (V150 L126 interaction)
  mutation (3868)..(3873): H130A R131E
  mutation (3892)..(3894): Expose T (L126 Y128 interaction)
  misc_feature (3895)..(3984): 6xGS Linker
  gene (3985)..(8088): Cas9(D10A)
  mutation (3985)..(3986): truncated 161
  sig_peptide (8101)..(8121): SV40 NLS
  terminator (8155)..(8342): ADH1 terminator
  rep_origin (8647)..(9102): f1 ori
  promoter (9402)..(9806): LEU2 promoter
  gene (9819)..(10913): LEU2
gacgaaagggcctcgtgatacgcctatttttataggttaatgtcatgataataatggtttcttaggacggatcgcttgcctgtaacttacacgcgcctcgtatcttttaatgatggaataatttgggaatttactctgtgtttatttatttttatgttttgtatttggattttagaaagtaaataaagaaggtagaagagttacggaatgaagaaaaaaaaataaacaaaggtttaaaaaatttcaacaaaaagcgtactttacatatatatttattagacaagaaaagcagattaaatagatatacattcgattaacgataagtaaaatgtaaaatcacaggattttcgtgtgtggtcttctacacagacaagatgaaacaattcggcattaatacctgagagcaggaagagcaagataaaaggtagtatttgttggcgatccccctagagtcttttacatcttcggaaaacaaaaactattttttctttaatttctttttttactttctatttttaatttatatatttatattaaaaaatttaaattataattatttttatagcacgtgatgaaaaggacccaggtggcacttttcggggaaatgtgcgcggaacccctatttgtttatttttctaaatacattcaaatatgtatccgctcatgagacaataaccctgataaatgcttcaataatattgaaaaaggaagagtatgagtattcaacatttccgtgtcgcccttattcccttttttgcggcattttgccttcctgtttttgctcacccagaaacgctggtgaaagtaaaagatgctgaagatcagttgggtgcacgagtgggttacatcgaactggatctcaacagcggtaagatccttgagagttttcgccccgaagaacgttttccaatgatgagcacttttaaagttctgctatgtggcgcggtattatcccgtattgacgccgggcaagagcaactcggtcgccgcatacactattctcagaatgacttggttgagtactcaccagtcacagaaaagcatcttacggatggcatgacagtaagagaattatgcagtgctgccataaccatgagtgataacactgcggccaacttacttctgacaacgatcggaggaccgaaggagctaaccgctttttttcacaacatgggggatcatgtaactcgccttgatcgttgggaaccggagctgaatgaagccataccaaacgacgagcgtgacaccacgatgcctgtagcaatggcaacaacgttgcgcaaactattaactggcgaactacttactctagcttcccggcaacaattaatagactggatggaggcggataaagttgcaggaccacttctgcgctcggcccttccggctggctggtttattgctgataaatctggagccggtgagcgtgggtctcgcggtatcattgcagcactggggccagatggtaagccctcccgtatcgtagttatctacacgacgggcagtcaggcaactatggatgaacgaaatagacagatcgctgagataggtgcctcactgattaagcattggtaactgtcagaccaagtttactcatatatactttagattgatttaaaacttcatttttaatttaaaaggatctaggtgaagatcctttttgataatctcatgaccaaaatcccttaacgtgagttttcgttccactgagcgtcagaccccgtagaaaagatcaaaggatcttcttgagatcctttttttctgcgcgtaatctgctgcttgcaaacaaaaaaaccaccgctaccagcggtggtttgtttgccggatcaagagctaccaactctttttccgaaggtaactggcttcagcagagcgcagataccaaatactgtccttctagtgtagccgtagttaggccaccacttcaagaactctgtagcaccgcctacatacctcgctctgctaatcctgttaccagtggctgctgccagtggcgataagtcgtgtcttaccgggttggactcaagacgatagttaccggataaggcgcagcggtcgggctgaacggggggttcgtgcacacagcccagcttggagcgaacgacctacaccgaactgagatacctacagcgtgagctatgagaaagcgccacgcttcccgaagggagaaaggcggacaggtatccggtaagcggcagggtcggaacaggagagcgcacgagggagcttccagggggaaacgcctggtatctttatagtcctgtcgggtttcgccacctctgacttgagcgtcgatttttgtgatgctcgtcaggggggcggagcctatggaaaaacgccagcaacgcggcctttttacggttcctggccttttgctggccttttgctcacatgttctttcctgcgttatcccctgattctgtggataaccgtattaccgcctttgagtgagctgataccgctcgccgcagccgaacgaccgagcgcagcgagtcagtgagcgaggaagcggaagagcgcccaatacgcaaaccgcctctccccgcgcgttggccgattcattaatgcagctggcacgacaggtttcccgactggaaagcgggcagtgagcgcaacgcaattaatgtgagttagctcactcattaggcaccccaggctttacactttatgcttccggctcgtatgttgtgtggaattgtgagcggataacaatttcacacaggaaacagctatgaccatgattacgccaagctcgaaattaaccctcactaaagggaacaaaagctggtaccgggcccgaattctctccttctcttaggtggcagagcaggtggagggtcgaccatactagtttcaaaaattcttactttttttttggatggacgcaaagaagtttaataatcatattacatggcattaccaccatatacatatccatatacatatccatatctaatcttacttatatgttgtggaaatgtaaagagccccattatcttagcctaaaaaaaccttctctttggaactttcagtaatacgcttaactgctcattgctatattgaagtacggattagaagccgccgagcgggtgacagccctccgaaggaagactctcctccgtgcgtcctcgtcttcaccggtcgcgttcctgaaacgcagatgtgcctcgcgccgcactgctccgaacaataaagattctacaatactagcttttatggttatgaagaggaaaaattggcagtaacctggccccacaaaccttcaaatgaacgaatcaaattaacaaccataggatgataatgcgattagttttttagccttatttctggggtaattaatcagcgaagcgatgatttttgatctattaacagatatataaatgcaaaaactgcataaccactttaactaatactttcaacattttcggtttgtattacttcttattcaaatgtaataaaagtatcaacaaaaaattgttaatatacctctatactttaacgtcaaggagaaaaaaccagcgctcttcgatgtcgcatagatgctacgttctctttgaattaaaacgacggggtgaacgtagagcgtgtttttggggctatgctgtgaataaaccacagagcgggacagaacgtggcattcacgccgaaatctttagcattagaaaagtcgaagaatacctgcgcgacaaccccggacaattcacgataaattggtactcatcctggagtccttgtgcagattgcgctgaaaagatcttagaatggtataaccaggagctgcgggggaacggccacactttgaaaatctgggcttgcaaactctattacgagaaaaatgcgaggaatcaaattgggctgtggaacctcagagataacggggttgggttgaatgtaggcggaggtggcagtggcgggggtggctcgggtgggggaggcagtggcggaggtggcagtggcgggggtggctcgggtgggggaggatccatggacaagaagtactccattgggctcgctatcggcacaaacagcgtcggttgggccgtcattacggacgagtacaaggtgccgagcaaaaaattcaaagttctgggcaataccgatcgccacagcataaagaagaacctcattggcgccctcctgttcgactccggggagacggccgaagccacgcggctcaaaagaacagcacggcgcagatatacccgcagaaagaatcggatctgctacctgcaggagatctttagtaatgagatggctaaggtggatgactctttcttccataggctggaggagtcctttttggtggaggaggataaaaagcacgagcgccacccaatctttggcaatatcgtggacgaggtggcgtaccatgaaaagtacccaaccatatatcatctgaggaagaagcttgtagacagtactgataaggctgacttgcggttgatctatctcgcgctggcgcatatgatcaaatttcggggacacttcctcatcgagggggacctgaacccagacaacagcgatgtcgacaaactctttatccaactggttcagacttacaatcagcttttcgaagagaacccgatcaacgcatccggagttgacgccaaagcaatcctgagcgctaggctgtccaaatcccggcggctcgaaaacctcatcgcacagctccctggggagaagaagaacggcctgtttggtaatcttatcgccctgtcactcgggctgacccccaactttaaatctaacttcgacctggccgaagatgccaagcttcaactgagcaaagacacctacgatgatgatctcgacaatctgctggcccagatcggcgaccagtacgcagacctttttttggcggcaaagaacctgtcagacgccattctgctgagtgatattctgcgagtgaacacggagatcaccaaagctccgctgagcgctagtatgatcaagcgctatgatgagcaccaccaagacttgactttgctgaaggcccttgtcagacagcaactgcctgagaagtacaaggaaattttcttcgatcagtctaaaaatggctacgccggatacattgacggcggagcaagccaggaggaattttacaaatttattaagcccatcttggaaaaaatggacggcaccgaggagctgctggtaaagcttaacagagaagatctgttgcgcaaacagcgcactttcgacaatggaagcatcccccaccagattcacctgggcgaactgcacgctatcctcaggcggcaagaggatttctacccctttttgaaagataacagggaaaagattgagaaaatcctcacatttcggataccctactatgtaggccccctcgcccggggaaattccagattcgcgtggatgactcgcaaatcagaagagaccatcactccctggaacttcgaggaagtcgtggataagggggcctctgcccagtccttcatcgaaaggatgactaactttgataaaaatctgcctaacgaaaaggtgcttcctaaacactctctgctgtacgagtacttcacagtttataacgagctcaccaaggtcaaatacgtcacagaagggatgagaaagccagcattcctgtctggagagcagaagaaagctatcgtggacctcctcttcaagacgaaccggaaagttaccgtgaaacagctcaaagaagactatttcaaaaagattgaatgtttcgactctgttgaaatcagcggagtggaggatcgcttcaacgcatccctgggaacgtatcacgatctcctgaaaatcattaaagacaaggacttcctggacaatgaggagaacgaggacattcttgaggacattgtcctcacccttacgttgtttgaagatagggagatgattgaagaacgcttgaaaacttacgctcatctcttcgacgacaaagtcatgaaacagctcaagaggcgccgatatacaggatgggggcggctgtcaagaaaactgatcaatgggatccgagacaagcagagtggaaagacaatcctggattttcttaagtccgatggatttgccaaccggaacttcatgcagttgatccatgatgactctctcacctttaaggaggacatccagaaagcacaagtttctggccagggggacagtcttcacgagcacatcgctaatcttgcaggtagcccagctatcaaaaagggaatactgcagaccgttaaggtcgtggatgaactcgtcaaagtaatgggaaggcataagcccgagaatatcgttatcgagatggcccgagagaaccaaactacccagaagggacagaagaacagtagggaaaggatgaagaggattgaagagggtataaaagaactggggtcccaaatccttaaggaacacccagttgaaaacacccagcttcagaatgagaagctctacctgtactacctgcagaacggcagggacatgtacgtggatcaggaactggacatcaatcggctctccgactacgacgtggatcatatcgtgccccagtcttttctcaaagatgattctattgataataaagtgttgacaagatccgataaaaatagagggaagagtgataacgtcccctcagaagaagttgtcaagaaaatgaaaaattattggcggcagctgctgaacgccaaactgatcacacaacggaagttcgataatctgactaaggctgaacgaggtggcctgtctgagttggataaagccggcttcatcaaaaggcagcttgttgagacacgccagatcaccaagcacgtggcccaaattctcgattcacgcatgaacaccaagtacgatgaaaatgacaaactgattcgagaggtgaaagttattactctgaagtctaagctggtctcagatttcagaaaggactttcagttttataaggtgagagagatcaacaattaccaccatgcgcatgatgcctacctgaatgcagtggtaggcactgcacttatcaaaaaatatcccaagcttgaatctgaatttgtttacggagactataaagtgtacgatgttaggaaaatgatcgcaaagtctgagcaggaaataggcaaggccaccgctaagtacttcttttacagcaatattatgaattttttcaagaccgagattacactggccaatggagagattcggaagcgaccacttatcgaaacaaacggagaaacaggagaaatcgtgtgggacaagggtagggatttcgcgacagtccggaaggtcctgtccatgccgcaggtgaacatcgttaaaaagaccgaagtacagaccggaggcttctccaaggaaagtatcctcccgaaaaggaacagcgacaagctgatcgcacgcaaaaaagattgggaccccaagaaatacggcggattcgattctcctacagtcgcttacagtgtactggttgtggccaaagtggagaaagggaagtctaaaaaactcaaaagcgtcaaggaactgctgggcatcacaatcatggagcgatcaagcttcgaaaaaaaccccatcgactttctcgaggcgaaaggatataaagaggtcaaaaaagacctcatcattaagcttcccaagtactctctctttgagcttgaaaacggccggaaacgaatgctcgctagtgcgggcgagctgcagaaaggtaacgagctggcactgccctctaaatacgttaatttcttgtatctggccagccactatgaaaagctcaaagggtctcccgaagataatgagcagaagcagctgttcgtggaacaacacaaacactaccttgatgagatcatcgagcaaataagcgaattctccaaaagagtgatcctcgccgacgctaacctcgataaggtgctttctgcttacaataagcacagggataagcccatcagggagcaggcagaaaacattatccacttgtttactctgaccaacttgggcgcgcctgcagccttcaagtacttcgacaccaccatagacagaaagcggtacacctctacaaaggaggtcctggacgccacactgattcatcagtcaattacggggctctatgaaacaagaatcgacctctctcagctcggtggagacagcagggctgaccccaagaagaagaggaaggtgtagtctagaggctccggataaggatcctaataagcgaatttcttatgatttatgatttttattattaaataagttataaaaaaaataagtgtatacaaattttaaagtgactcttaggttttaaaacgaaaattcttattcttgagtaactctttcctgtaggtcaggttgctttctcaggtatagcatgaggtcgctcttattgaccacacctctaccggcatgccgagcaaatgcctgcaaatcgctcccgggcaaaaaaccccctcaagacccgtttagaggccccaaggggttatgctatgcataccaagcttccgcggtggagctccaattcgccctatagtgagtcgtattacaattcactggccgtcgttttacaacgtcgtgactgggaaaaccctggcgttacccaacttaatcgccttgcagcacatccccccttcgccagctggcgtaatagcgaagaggcccgcaccgatcgcccttcccaacagttgcgcagcctgaatggcgaatggcgcgacgcgccctgtagcggcgcattaagcgcggcgggtgtggtggttacgcgcagcgtgaccgctacacttgccagcgccctagcgcccgctcctttcgctttcttcccttcctttctcgccacgttcgccggctttccccgtcaagctctaaatcgggggctccctttagggttccgatttagtgctttacggcacctcgaccccaaaaaacttgattagggtgatggttcacgtagtgggccatcgccctgatagacggtttttcgccctttgacgttggagtccacgttctttaatagtggactcttgttccaaactggaacaacactcaaccctatctcggtctattcttttgatttataagggattttgccgatttcggcctattggttaaaaaatgagctgatttaacaaaaatttaacgcgaattttaacaaaatattaacgtttacaatttcctgatgcggtattttctccttacgcatctgtgcggtatttcacaccgcatatcgaccctcgaggagaacttctagtatatccacatacctaatattattgccttattaaaaatggaatcggaacaattacatcaaaatccacattctcttcaaaatcaattgtcctgtacttccttgttcatgtgtgttcaaaaacgttatatttataggataattatactctatttctcaacaagtaattggttgtttggccgagcggtctaaggcgcctgattcaagaaatatcttgaccgcagttaactgtgggaatactcaggtatcgtaagatgcaagagttcgaatctcttagcaaccattatttttttcctcaacataacgagaacacacaggggcgctatcgcacagaatcaaattcgatgactggaaattttttgttaatttcagaggtcgcctgacgcatatacctttttcaactgaaaaattgggagaaaaaggaaaggtgagaggccggaaccggcttttcatatagaatagagaagcgttcatgactaaatgcttgcatcacaatacttgaagttgacaatattatttaaggacctattgttttttccaataggtggttagcaatcgtcttactttctaacttttcttaccttttacatttcagcaatatatatatatatttcaaggatataccattctaatgtctgcccctatgtctgcccctaagaagatcgtcgttttgccaggtgaccacgttggtcaagaaatcacagccgaagccattaaggttcttaaagctatttctgatgttcgttccaatgtcaagttcgatttcgaaaatcatttaattggtggtgctgctatcgatgctacaggtgtcccacttccagatgaggcgctggaagcctccaagaaggttgatgccgttttgttaggtgctgtgggtggtcctaaatggggtaccggtagtgttagacctgaacaaggtttactaaaaatccgtaaagaacttcaattgtacgccaacttaagaccatgtaactttgcatccgactctcttttagacttatctccaatcaagccacaatttgctaaaggtactgacttcgttgttgtcagagaattagtgggaggtatttactttggtaagagaaaggaagacgatggtgatggtgtcgcttgggatagtgaacaatacaccgttccagaagtgcaaagaatcacaagaatggccgctttcatggccctacaacatgagccaccattgcctatttggtccttggataaagctaatgttttggcctcttcaagattatggagaaaaactgtggaggaaaccatcaagaacgaattccctacattgaaggttcaacatcaattgattgattctgccgccatgatcctagttaagaacccaacccacctaaatggtattataatcaccagcaacatgtttggtgatatcatctccgatgaagcctccgttatcccaggttccttgggtttgttgccatctgcgtccttggcctctttgccagacaagaacaccgcatttggtttgtacgaaccatgccacggttctgctccagatttgccaaagaataaggttgaccctatcgccactatcttgtctgctgcaatgatgttgaaattgtcattgaacttgcctgaagaaggtaaggccattgaagatgcagttaaaaaggttttggatgcaggtatcagaactggtgatttaggtggttccaacagtaccaccgaagtcggtgatgctgtcgccgaagaagttaagaaaatccttgcttaaaaagattctctttttttatgatatttgtacataaactttataaatgaaattcataatagaaacgacacgaaattacaaaatggaatatgttcatagggtagacgaaactatatacgcaatctacatacatttatcaagaaggagaaaaaggaggatagtaaaggaatacaggtaagcaaattgatactaatggctcaacgtgataaggaaaaagaattgcactttaacattaatattgacaaggaggagggcaccacacaaaaagttaggtgtaacagaaaatcatgaaactacgattcctaatttgatattggaggattttctctaaaaaaaaaaaaatacaacaaataaaaaacactcaatgacctgaccatttgatggagtttaagtcaataccttcttgaaccatttcccataatggtgaaagttccctcaagaattttactctgtcagaaacggccttacgacgtagtcgatatggtgcactctcagtacaatctgctctgatgccgcatagttaagccagccccgacacccgccaacacccgctgacgcgccctgacgggcttgtctgctcccggcatccgcttacagacaagctgtgaccgtctccgggagctgcatgtgtcagaggttttcaccgtcatcaccgaaacgcgcga

SEQ ID NO: 14 - DNA, 11801 bp, Artificial Sequence
  full-length sequence of vector V5679
  rep_origin (70)..(573): CEN/ARS
  promoter (610)..(714): AmpR promoter
  gene (715)..(1575): AmpR
  rep_origin (1746)..(2334): ori
  promoter (2658)..(2688): lac promoter
  misc_feature (2696)..(2712): lac operator
  promoter (2853)..(3517): GAL1,10 promoter
  misc_feature (3069)..(3186): UAS
  gene (3502)..(6681): nCas9(D10A)
  mutation (3547)..(3549): D10A for Nuclease deficient
  misc_feature (6682)..(6688): GS linker insert
  misc_feature (6689)..(6702): Linker
  misc_feature (6703)..(6768): 3xFLAG
  gene (6775)..(7398): PmCDA1
  misc_feature (7419)..(7431): GS linker insert
  gene (7432)..(8409): nCas9(D10A)
  sig_peptide (8386)..(8406): SV40 NLS
  terminator (8422)..(8669): CYC1 terminator
  rep_origin (8873)..(9328): f1 ori
  promoter (9628)..(10032): LEU2 promoter
  gene (10045)..(11139): LEU2
gacgaaagggcctcgtgatacgcctatttttataggttaatgtcatgataataatggtttcttaggacggatcgcttgcctgtaacttacacgcgcctcgtatcttttaatgatggaataatttgggaatttactctgtgtttatttatttttatgttttgtatttggattttagaaagtaaataaagaaggtagaagagttacggaatgaagaaaaaaaaataaacaaaggtttaaaaaatttcaacaaaaagcgtactttacatatatatttattagacaagaaaagcagattaaatagatatacattcgattaacgataagtaaaatgtaaaatcacaggattttcgtgtgtggtcttctacacagacaagatgaaacaattcggcattaatacctgagagcaggaagagcaagataaaaggtagtatttgttggcgatccccctagagtcttttacatcttcggaaaacaaaaactattttttctttaatttctttttttactttctatttttaatttatatatttatattaaaaaatttaaattataattatttttatagcacgtgatgaaaaggacccaggtggcacttttcggggaaatgtgcgcggaacccctatttgtttatttttctaaatacattcaaatatgtatccgctcatgagacaataaccctgataaatgcttcaataatattgaaaaaggaagagtatgagtattcaacatttccgtgtcgcccttattcccttttttgcggcattttgccttcctgtttttgctcacccagaaacgctggtgaaagtaaaagatgctgaagatcagttgggtgcacgagtgggttacatcgaactggatctcaacagcggtaagatccttgagagttttcgccccgaagaacgttttccaatgatgagcacttttaaagttctgctatgtggcgcggtattatcccgtattgacgccgggcaagagcaactcggtcgccgcatacactattctcagaatgacttggttgagtactcaccagtcacagaaaagcatcttacggatggcatgacagtaagagaattatgcagtgctgccataaccatgagtgataacactgcggccaacttacttctgacaacgatcggaggaccgaaggagctaaccgcttttttgcacaacatgggggatcatgtaactcgccttgatcgttgggaaccggagctgaatgaagccataccaaacgacgagcgtgacaccacgatgcctgtagcaatggcaacaacgttgcgcaaactattaactggcgaactacttactctagcttcccggcaacaattaatagactggatggaggcggataaagttgcaggaccacttctgcgctcggcccttccggctggctggtttattgctgataaatctggagccggtgagcgtgggtctcgcggtatcattgcagcactggggccagatggtaagccctcccgtatcgtagttatctacacgacggggagtcaggcaactatggatgaacgaaatagacagatcgctgagataggtgcctcactgattaagcattggtaactgtcagaccaagtttactcatatatactttagattgatttaaaacttcatttttaatttaaaaggatctaggtgaagatcctttttgataatctcatgaccaaaatcccttaacgtgagttttcgttccactgagcgtcagaccccgtagaaaagatcaaaggatcttcttgagatcctttttttctgcgcgtaatctgctgcttgcaaacaaaaaaaccaccgctaccagcggtggtttgtttgccggatcaagagctaccaactctttttccgaaggtaactggcttcagcagagcgcagataccaaatactgtccttctagtgtagccgtagttaggccaccacttcaagaactctgtagcaccgcctacatacctcgctctgctaatcctgttaccagtggctgctgccagtggcgataagtcgtgtcttaccgggttggactcaagacgatagttaccggataaggcgcagcggtcgggctgaacggggggttcgtgcacacagcccagcttggagcgaacgacctacaccgaactgagatacctacagcgtgagctatgagaaagcgccacgcttcccgaagggagaaaggcggacaggtatccggtaagcggcagggtcggaacaggagagcgcacgagggagcttccagggggaaacgcctggtatctttatagtcctgtcgggtttcgccacctctgacttgagcgtcgatttttgtgatgctcgtcaggggggcggagcctatggaaaaacgccagcaacgcggcctttttacggttcctggccttttgctggccttttgctcacatgttctttcctgcgttatcccctgattctgtggataaccgtattaccgcctttgagtgagctgataccgctcgccgcagccgaacgaccgagcgcagcgagtcagtgagcgaggaagcggaagagcgcccaatacgcaaaccgcctctccccgcgcgttggccgattcattaatgcagctggcacgacaggtttcccgactggaaagcgggcagtgagcgcaacgcaattaatgtgagttacctcactcattaggcaccccaggctttacactttatgcttccggctcctatgttgtgtggaattgtgagcggataacaatttcacacaggaaacagctatgaccatgattacgccaagctcggaattaaccctcactaaagggaacaaaagctgggtaccgggcccgaattctctccttctcttaggtggcagagcaggtggagggtcgaccatactagtttcaaaaattcttactttttttttggatggacgcaaagaagtttaataatcatattacatggcattaccaccatatacatatccatatacatatccatatctaatcttacttatatgttgtggaaatgtaaagagccccattatcttagcctaaaaaaaccttctctttggaactttcagtaatacgcttaactgctcattgctatattgaagtacggattagaagccgccgagcgggtgacagccctccgaaggaagactctcctccgtgcgtcctcgtcttcaccggtcgcgttcctgaaacgcagatgtgcctcgcgccgcactgctccgaacaataaagattctacaatactagcttttatggttatgaagaggaaaaattggcagtaacctggccccacaaaccttcaaatgaacgaatcaaattaacaaccataggatgataatgcgattagttttttagccttatttctggggtaattaatcagcgaagcgatgatttttgatctattaacagatatataaatgcaaaaactgcataaccactttaactaatactttcaacattttcggtttgtattacttcttattcaaatgtaataaaagtatcaacaaaaaattgttaatatacctctatactttaacgtcaaggagaaaaaacccatggacaagaagtactccattgggctcgctatcggcacaaacagcgtcggttgggccgtcattacggacgagtacaaggtgccgagcaaaaaattcaaagttctgggcaataccgatcgccacagcataaagaagaacctcattggcgccctcctgttcgactccggggagacggccgaagccacgcggctcaaaagaacagcacggcgcagatatacccgcagaaagaatcggatctgctacctgcaggagatctttagtaatgagatggctaaggtggatgactctttcttccataggctggaggagtcctttttggtggaggaggataaaaagcacgagcgccacccaatctttggcaatatcgtggacgaggtggcgtaccatgaaaagtacccaaccatatatcatctgaggaagaagcttgtagacagtactgataaggctgacttgcggttgatctatctcgcgctggcgcatatgatcaaatttcggggacacttcctcatcgagggggacctgaacccagacaacagcgatgtcgacaaactctttatccaactggttcagacttacaatcagcttttcgaagagaacccgatcaacgcatccggagttgacgccaaagcaatcctgagcgctaggctgtccaaatcccggcggctcgaaaacctcatcgcacagctccctggggagaagaagaacggcctgtttggtaatcttatcgccctgtcactcgggctgacccccaactttaaatctaacttcgacctggccgaagatgccaagcttcaactgagcaaagacacctacgatgatgatctcgacaatctgctggcccagatcggcgaccagtacgcagacctttttttggcggcaaagaacctgtcagacgccattctgctgagtgatattctgcgagtgaacacggagatcaccaaagctccgctgagcgctagtatgatcaagcgctatgatgagcaccaccaagacttgactttgctgaaggcccttgtcagacagcaactgcctgagaagtacaaggaaattttcttcgatcagtctaaaaatggctacgccggatacattgacggcggagcaagccaggaggaattttacaaatttattaagcccatcttggaaaaaatggacggcaccgaggagctgctggtaaagcttaacagagaagatctgttgcgcaaacagcgcactttcgacaatggaagcatcccccaccagattcacctgggcgaactgcacgctatcctcaggcggcaagaggatttctacccctttttgaaagataacagggaaaagattgagaaaatcctcacatttcggataccctactatgtaggccccctcgcccggggaaattccagattcgcgtggatgactcgcaaatcagaagagaccatcactccctggaacttcgaggaagtcgtggataagggggcctctgcccagtccttcatcgaaaggatgactaactttgataaaaatctgcctaacgaaaaggtgcttcctaaacactctctgctgtacgagtacttcacagtttataacgagctcaccaaggtcaaatacgtcacagaagggatgagaaagccagcattcctgtctggagagcagaagaaagctatcgtggacctcctcttcaagacgaaccggaaagttaccgtgaaacagctcaaagaagactatttcaaaaagattgaatgtttcgactctgttgaaatcagcggagtggaggatcgcttcaacgcatccctgggaacgtatcacgatctcctgaaaatcattaaagacaaggacttcctggacaatgaggagaacgaggacattcttgaggacattgtcctcacccttacgttgtttgaagatagggagatgattgaagaacgcttgaaaacttacgctcatctcttcgacgacaaagtcatgaaacagctcaagaggcgccgatatacaggatgggggcggctgtcaagaaaactgatcaatgggatccgagacaagcagagtggaaagacaatcctggattttcttaagtccgatggatttgccaaccggaacttcatgcagttgatccatgatgactctctcacctttaaggaggacatccagaaagcacaagtttctggccagggggacagtcttcacgagcacatcgctaatcttgcaggtagcccagctatcaaaaagggaatactgcagaccgttaaggtcgtggatgaactcgtcaaagtaatgggaaggcataagcccgagaatatcgttatcgagatggcccgagagaaccaaactacccagaagggacagaagaacagtagggaaaggatgaagaggattgaagagggtataaaagaactggggtcccaaatccttaaggaacacccagttgaaaacacccagcttcagaatgagaagctctacctgtactacctgcagaacggcagggacatgtacgtggatcaggaactggacatcaatcggctctccgactacgacgtggatcatatcgtgccccagtcttttctcaaagatgattctattgataataaagtgttgacaagatccgataaaaatagagggaagagtgataacgtcccctcagaagaagttgtcaagaaaatgaaaaattattggcggcagctgctgaacgccaaactgatcacacaacggaagttcgataatctgactaaggctgaacgaggtggcctgtctgagttggataaagccggcttcatcaaaaggcagcttgttgagacacgccagatcaccaagcacgtggcccaaattctcgattcacgcatgaacaccaagtacgatgaaaatgacaaactgattcgagaggtgaaagttattactctgaagtctaagctggtctcagatttcagaaaggactttcagttttataaggtgagagagatcaacaattaccaccatgcgcatgatgcctacctgaatgcagtggtaggcactgcacttatcaaaaaatatcccaagcttgaatctgaatttgtttacggagactataaagtgtacgatgttaggaaaatgatcgcaaagtctgagcaggaaataggcaaggccaccgctaagtacttcttttacagcaatattatgaattttttcaagaccgagattacactggccaatggtggagctagcggttccggagactataaggaccacgacggagactacaaggatcatgatattgattacaaagacgatgacgataagtctaggatgaccgacgctgagtacgtgagaatccatgagaagttggacatctacacgtttaagaaacagtttttcaacaacaaaaaatccgtgtcgcatagatgctacgttctctttgaattaaaacgacggggtgaacgtagagcgtgtttttggggctatgctgtgaataaaccacagagcgggacagaacgtggcattcacgccgaaatctttagcattagaaaagtcgaagaatacctgcgcgacaaccccggacaattcacgataaattggtactcatcctggagtccttgtgcagattgcgctgaaaagatcttagaatggtataaccaggagctgcgggggaacggccacactttgaaaatctgggcttgcaaactctattacgagaaaaatgcgaggaatcaaattgggctgtggaacctcagagataacggggttgggttgaatgtaatggtaagtgaacactaccaatgttgcaggaaaatattcatccaatcgtcgcacaatcaattgaatgagaatagatggcttgagaagactttgaagcgagctgaaaaacgacggagcgagttgtccattatgattcaggtaaaaatactccacaccactaagagtcctgctgttggcggaggcggtagcgacgtcggtggaggttcaggagagattcggaagcgaccacttatcgaaacaaacggagaaacaggagaaatcgtgtgggacaagggtagggatttcgcgacagtccggaaggtcctgtccatgccgcaggtgaacatcgttaaaaagaccgaagtacagaccggaggcttctccaaggaaagtatcctcccgaaaaggaacagcgacaagctgatcgcacgcaaaaaagattgggaccccaagaaatacggcggattcgattctcctacagtcgcttacagtgtactggttgtggccaaagtggagaaagggaagtctaaaaaactcaaaagcgtcaaggaactgctgggcatcacaatcatggagcgatcaagcttcgaaaaaaaccccatcgactttctcgaggcgaaaggatataaagaggtcaaaaaagacctcatcattaagcttcccaagtactctctctttgagcttgaaaacggccggaaacgaatgctcgctagtgcgggcgagctgcagaaaggtaacgagctggcactgccctctaaatacgttaatttcttgtatctggccagccactatgaaaagctcaaagggtctcccgaagataatgagcagaagcagctgttcgtggaacaacacaaacactaccttgatgagatcatcgagcaaataagcgaattctccaaaagagtgatcctcgccgacgctaacctcgataaggtgctttctgcttacaataagcacagggataagcccatcagggagcaggcagaaaacattatccacttgtttactctgaccaacttgggcgcgcctgcagccttcaagtacttcgacaccaccatagacagaaagcggtacacctctacaaaggaggtcctggacgccacactgattcatcagtcaattacggggctctatgaaacaagaatcgacctctctcagctcggtggagacagcagggctgaccccaagaagaagaggaaggtgtgatctcttctcgagtcatgtaattagttatgtcacgcttacattcacgccctccccccacatccgctctaaccgaaaaggaaggagttagacaacctgaagtctaggtccctatttatttttttatagttatgttagtattaagaacgttatttatatttcaaatttttcttttttttctgtacagacgcgtgtacgcatgtaacattatactgaaaaccttgcttgagaaggttttgggacgctcgaaggctttaatttgcggccggtacccaattcgccctatagtgagtcgtattacgcgcgctcactggccgtcgttttacaacgtcgtgactgggaaaaccctggcgttacccaacttaatcgccttgcagcacatccccctttcgccagctggcgtaatagcgaagaggcccgcaccgatcgcccttcccaacagttgcgcagcctgaatggcgaatggacgcgccctgtagcggcgcattaagcgcggcgggtgtggtggttacgcgcagcgtgaccgctacacttgccagcgccctagcgcccgctcctttcgctttcttcccttcctttctcgccacgttcgccggctttccccgtcaagctctaaatcgggggctccctttagggttccgatttagtgctttacggcacctcgaccccaaaaaacttgattagggtgatggttcacgtagtgggccatcgccctgatagacggtttttcgccctttgacgttggagtccacgttctttaatagtggactcttgttccaaactggaacaacactcaaccctatctcggtctattcttttgatttataagggattttgccgatttcggcctattggttaaaaaatgagctgatttaacaaaaatttaacgcgaattttaacaaaatattaacgtttacaatttcctgatgcggtattttctccttacgcatctgtgcggtatttcacaccgcatatcgacggtcgaggagaacttctagtatatccacatacctaatattattgccttattaaaaatggaatcccaacaattacatcaaaatccacattctcttcaaaatcaattgtcctgtacttccttgttcatgtgtgttcaaaaacgttatatttataggataattatactctatttctcaacaagtaattggttgtttggccgagcggtctaaggcgcctgattcaagaaatatcttgaccgcagttaactgtgggaatactcaggtatcgtaagatgcaagagttcgaatctcttagcaaccattatttttttcctcaacataacgagaacacacaggggcgctatcgcacagaatcaaattcgatgactggaaattttttgttaatttcagaggtcgcctgacgcatatacctttttcaactgaaaaattgggagaaaaaggaaaggtgagaggccggaaccggcttttcatatagaatagagaagcgttcatgactaaatgcttgcatcacaatacttgaagttgacaatattatttaaggacctattgttttttccaataggtggttagcaatcgtcttactttctaacttttcttaccttttacatttcagcaatatatatatatatttcaaggatataccattctaatgtctgcccctatgtctgcccctaagaagatcgtcgttttgccaggtgaccacgttggtcaagaaatcacagccgaagccattaaggttcttaaagctatttctgatgttcgttccaatgtcaagttcgatttcgaaaatcatttaattggtggtgctgctatcgatgctacaggtgtcccacttccagatgaggcgctggaagcctccaagaaggttgatgccgttttgttaggtgctgtgggtggtcctaaatggggtaccggtagtgttagacctgaacaaggtttactaaaaatccgtaaagaacttcaattgtacgccaacttaagaccatgtaactttgcatccgactctcttttagacttatctccaatcaagccacaatttgctaaaggtactgacttcgttgttgtcagagaattagtgggaggtatttactttggtaagagaaaggaagacgatggtgatggtgtcgcttgggatagtgaacaatacaccgttccagaagtgcaaagaatcacaagaatggccgctttcatggccctacaacatgagccaccattgcctatttggtccttggataaagctaatgttttggcctcttcaagattatggagaaaaactgtggaggaaaccatcaagaacgaattccctacattgaaggttcaacatcaattgattgattctgccgccatgatcctagttaagaacccaacccacctaaatggtattataatcaccagcaacatgtttggtgatatcatctccgatgaagcctccgttatcccaggttccttgggtttgttgccatctgcgtccttggcctctttgccagacaagaacaccgcatttggtttgtacgaaccatgccacggttctgctccagatttgccaaagaataaggtcaaccctatcgccactatcttgtctgctgcaatgatgttgaaattgtcattgaacttgcctgaagaaggtaaggccattgaagatgcagttaaaaaggttttggatgcaggtatcagaactggtgatttaggtggttccaacagtaccaccgaagtcggtgatgctgtcgccgaagaagttaagaaaatccttgcttaaaaagattctctttttttatgatatttgtacataaactttataaatgaaattcataatagaaacgacacgaaattacaaaatggaatatgttcatagggtagacgaaactatatacgcaatctacatacatttatcaagaaggagaaaaaggaggatgtaaaggaatacaggtaagcaaattgatactaatggctcaacgtgataaggaaaaagaattgcactttaacattaatattgacaaggaggagggcaccacacaaaaagttaggtgtaacagaaaatcatgaaactatgattcctaatttatatattggaggattttctctaaaaaaaaaaaaatacaacaaataaaaaacactcaatgacctgaccatttgatggagtttaagtcaataccttcttgaaccatttcccataatggtgaaagttccctcaagaattttactctgtcagaaacggccttacgacgtagtcgatatggtgcactctcagtacaatctgctctgatgccgcatagttaagccagccccgacacccgccaacacccgctgacgcgccctgacgggcttgtctgctcccggcatccgcttacagacaagctgtgaccgtctccgggagctgcatgtgtcagaggttttcaccgtcatcaccgaaacgcgcga

SEQ ID NO: 15 - DNA, 11447 bp, Artificial Sequence
  full-length sequence of vector pAL047
  rep_origin (70)..(573): CEN/ARS
  promoter (610)..(714): AmpR promoter
  gene (715)..(1575): AmpR
  rep_origin (1746)..(2334): ori
  promoter (2658)..(2688): lac promoter
  misc_feature (2696)..(2712): lac operator
  promoter (2853)..(3517): GAL1,10 promoter
  gene (3520)..(6681): nCas9(D10A)
  mutation (3547)..(3549): D10A for Nuclease deficient
  gene (6682)..(7044): PmCDA1
  misc_feature (6790)..(6897): Catalytic Domain
  mutation (6958)..(6960): W122E
  mutation (6970)..(6972): Expsose N (V150 Y128 interaction)
  mutation (6976)..(6978): Expose Q (V150 L126 interaction)
  mutation (6976)..(6978): Expose Y to D
  mutation (7000)..(7002): Expose I to E
  mutation (7009)..(7011): W139Q
  mutation (7018)..(7023): H130A R131E
  mutation (7042)..(7044): Expose T (L126 Y128 interaction)
  misc_feature (7045)..(7070): 6xGS Linker
  misc_feature (7065)..(7077): GS linker insert
  gene (7078)..(8055): nCas9(D10A)
  sig_peptide (8032)..(8052): SV40 NLS
  terminator (8068)..(8315): CYC1 terminator
  rep_origin (8519)..(8974): f1 ori
  promoter (9274)..(9678): LEU2 promoter
  gene (9691)..(10785): LEU2
gacgaaagggcctcgtgatacgcctatttttataggttaatgtcatgataataatggtttcttaggacggatcgcttgcctgtaacttacacgcgcctcgtatcttttaatgatggaataatttgggaatttactctgtgtttatttatttttatgttttgtatttggattttagaaagtaaataaagaaggtagaagagttacggaatgaagaaaaaaaaataaacaaaggtttaaaaaatttcaacaaaaagcgtactttacatatatatttattagacaagaaaagcagattaaatagatatacattcgattaacgataagtaaaatgtaaaatcacaggattttcgtgtgtggtcttctacacagacaagatgaaacaattcggcattaatacctgagagcaggaagagcaagataaaaggtagtatttgttggcgatccccctagagtcttttacatcttcggaaaacaaaaactattttttctttaatttctttttttactttctatttttaatttatatatttatattaaaaaatttaaattataattatttttatagcacgtgatgaaaaggacccaggtggcacttttcggggaaatgtgcgcggaacccctatttgtttatttttctaaatacattcaaatatgtatccgctcatgagacaataaccctgataaatgcttcaataatattgaaaaaggaagagtatgagtattcaacatttccgtgtcgcccttattcccttttttgcggcattttgccttcctgtttttgctcacccagaaacgctggtgaaagtaaaagatgctgaagatcagttgggtgcacgagtgggttacatcgaactggatctcaacagcggtaagatccttgagagttttcgccccgaagaacgttttccaatgatgagcacttttaaagttctgctatgtggcgcggtattatcccgtattgacgccgggcaagagcaactcggtcgccgcatacactattctcagaatgacttggttgagtactcaccagtcacagaaaagcatcttacggatggcatgacagtaagagaattatgcagtgctgccataaccatgagtgataacactgcggccaacttacttctgacaacgatcggaggaccgaaggagctaaccgcttttttgcacaacatgggggatcatgtaactcgccttgatcgttgggaaccggagctgaatgaagccataccaaacgacgagcgtgacaccacgatgcctgtagcaatggcaacaacgttgcgcaaactattaactggcgaactacttactctagcttcccggcaacaattaatagactggatggaggcggataaagttgcaggaccacttctgcgctcggcccttccggctggctggtttattgctgataaatctggagccggtgagcgtgggtctcgcggtatcattgcagcactggggccagatggtaagccctcccgtatcgtagttatctacacgacggggagtcaggcaactatggatgaacgaaatagacagatcgctgagataggtgcctcactgattaagcattggtaactgtcagaccaagtttactcatatatactttagattgatttaaaacttcatttttaatttaaaaggatctaggtgaagatcctttttgataatctcatgaccaaaatcccttaacgtgagttttcgttccactgagcgtcagaccccgtagaaaagatcaaaggatcttcttgagatcctttttttctgcgcgtaatctgctgcttgcaaacaaaaaaaccaccgctaccagcggtggtttgtttgccggatcaagagctaccaactctttttccgaaggtaactggcttcagcagagcgcagataccaaatactgtccttctagtgtagccgtagttaggccaccacttcaagaactctgtagcaccgcctacatacctcgctctgctaatcctgttaccagtggctgctgccagtggcgataagtcgtgtcttaccgggttggactcaagacgatagttaccggataaggcgcagcggtcgggctgaacggggggttcgtgcacacagcccagcttggagcgaacgacctacaccgaactgagatacctacagcgtgagctatgagaaagcgccacgcttcccgaagggagaaaggcggacaggtatccggtaagcggcagggtcggaacaggagagcgcacgagggagcttccagggggaaacgcctggtatctttatagtcctgtcgggtttcgccacctctgacttgagcgtcgatttttgtgatgctcgtcaggggggcggagcctatggaaaaacgccagcaacgcggcctttttacggttcctggccttttgctggccttttgctcacatgttctttcctgcgttatcccctgattctgtggataaccgtattaccgcctttgagtgagctgataccgctcgccgcagccgaacgaccgagcgcagcgagtcagtgagcgaggaagcggaagagcgcccaatacgcaaaccgcctctccccgcgcgttggccgattcattaatgcagctggcacgacaggtttcccgactggaaagcgggcagtgagcgcaacgcaattaatgtgagttacctcactcattaggcaccccaggctttacactttatgcttccggctcctatgttgtgtggaattgtgagcggataacaatttcacacaggaaacagctatgaccatgattacgccaagctcggaattaaccctcactaaagggaacaaaagctgggtaccgggcccgaattctctccttctcttaggtggcagagcaggtggagggtcgaccatactagtttcaaaaattcttactttttttttggatggacgcaaagaagtttaataatcatattacatggcattaccaccatatacatatccatatacatatccatatctaatcttacttatatgttgtggaaatgtaaagagccccattatcttagcctaaaaaaaccttctctttggaactttcagtaatacgcttaactgctcattgctatattgaagtacggattagaagccgccgagcgggtgacagccctccgaaggaagactctcctccgtgcgtcctcgtcttcaccggtcgcgttcctgaaacgcagatgtgcctcgcgccgcactgctccgaacaataaagattctacaatactagcttttatggttatgaagaggaaaaattggcagtaacctggccccacaaaccttcaaatgaacgaatcaaattaacaaccataggatgataatgcgattagttttttagccttatttctggggtaattaatcagcgaagcgatgatttttgatctattaacagatatataaatgcaaaaactgcataaccactttaactaatactttcaacattttcggtttgtattacttcttattcaaatgtaataaaagtatcaacaaaaaattgttaatatacctctatactttaacgtcaaggagaaaaaacccatggacaagaagtactccattgggctcgctatcggcacaaacagcgtcggttgggccgtcattacggacgagtacaaggtgccgagcaaaaaattcaaagttctgggcaataccgatcgccacagcataaagaagaacctcattggcgccctcctgttcgactccggggagacggccgaagccacgcggctcaaaagaacagcacggcgcagatatacccgcagaaagaatcggatctgctacctgcaggagatctttagtaatgagatggctaaggtggatgactctttcttccataggctggaggagtcctttttggtggaggaggataaaaagcacgagcgccacccaatctttggcaatatcgtggacgaggtggcgtaccatgaaaagtacccaaccatatatcatctgaggaagaagcttgtagacagtactgataaggctgacttgcggttgatctatctcgcgctggcgcatatgatcaaatttcggggacacttcctcatcgagggggacctgaacccagacaacagcgatgtcgacaaactctttatccaactggttcagacttacaatcagcttttcgaagagaacccgatcaacgcatccggagttgacgccaaagcaatcctgagcgctaggctgtccaaatcccggcggctcgaaaacctcatcgcacagctccctggggagaagaagaacggcctgtttggtaatcttatcgccctgtcactcgggctgacccccaactttaaatctaacttcgacctggccgaagatgccaagcttcaactgagcaaagacacctacgatgatgatctcgacaatctgctggcccagatcggcgaccagtacgcagacctttttttggcggcaaagaacctgtcagacgccattctgctgagtgatattctgcgagtgaacacggagatcaccaaagctccgctgagcgctagtatgatcaagcgctatgatgagcaccaccaagacttgactttgctgaaggcccttgtcagacagcaactgcctgagaagtacaaggaaattttcttcgatcagtctaaaaatggctacgccggatacattgacggcggagcaagccaggaggaattttacaaatttattaagcccatcttggaaaaaatggacggcaccgaggagctgctggtaaagcttaacagagaagatctgttgcgcaaacagcgcactttcgacaatggaagcatcccccaccagattcacctgggcgaactgcacgctatcctcaggcggcaagaggatttctacccctttttgaaagataacagggaaaagattgagaaaatcctcacatttcggataccctactatgtaggccccctcgcccggggaaattccagattcgcgtggatgactcgcaaatcagaagagaccatcactccctggaacttcgaggaagtcgtggataagggggcctctgcccagtccttcatcgaaaggatgactaactttgataaaaatctgcctaacgaaaaggtgcttcctaaacactctctgctgtacgagtacttcacagtttataacgagctcaccaaggtcaaatacgtcacagaagggatgagaaagccagcattcctgtctggagagcagaagaaagctatcgtggacctcctcttcaagacgaaccggaaagttaccgtgaaacagctcaaagaagactatttcaaaaagattgaatgtttcgactctgttgaaatcagcggagtggaggatcgcttcaacgcatccctgggaacgtatcacgatctcctgaaaatcattaaagacaaggacttcctggacaatgaggagaacgaggacattcttgaggacattgtcctcacccttacgttgtttgaagatagggagatgattgaagaacgcttgaaaacttacgctcatctcttcgacgacaaagtcatgaaacagctcaagaggcgccgatatacaggatgggggcggctgtcaagaaaactgatcaatgggatccgagacaagcagagtggaaagacaatcctggattttcttaagtccgatggatttgccaaccggaacttcatgcagttgatccatgatgactctctcacctttaaggaggacatccagaaagcacaagtttctggccagggggacagtcttcacgagcacatcgctaatcttgcaggtagcccagctatcaaaaagggaatactgcagaccgttaaggtcgtggatgaactcgtcaaagtaatgggaaggcataagcccgagaatatcgttatcgagatggcccgagagaaccaaactacccagaagggacagaagaacagtagggaaaggatgaagaggattgaagagggtataaaagaactggggtcccaaatccttaaggaacacccagttgaaaacacccagcttcagaatgagaagctctacctgtactacctgcagaacggcagggacatgtacgtggatcaggaactggacatcaatcggctctccgactacgacgtggatcatatcgtgccccagtcttttctcaaagatgattctattgataataaagtgttgacaagatccgataaaaatagagggaagagtgataacgtcccctcagaagaagttgtcaagaaaatgaaaaattattggcggcagctgctgaacgccaaactgatcacacaacggaagttcgataatctgactaaggctgaacgaggtggcctgtctgagttggataaagccggcttcatcaaaaggcagcttgttgagacacgccagatcaccaagcacgtggcccaaattctcgattcacgcatgaacaccaagtacgatgaaaatgacaaactgattcgagaggtgaaagttattactctgaagtctaagctggtctcagatttcagaaaggactttcagttttataaggtgagagagatcaacaattaccaccatgcgcatgatgcctacctgaatgcagtggtaggcactgcacttatcaaaaaatatcccaagcttgaatctgaatttgtttacggagactataaagtgtacgatgttaggaaaatgatcgcaaagtctgagcaggaaataggcaaggccaccgctaagtacttcttttacagcaatattatgaattttttcaagaccgagattacactggccaattcgcatagatgctacgttctctttgaattaaaacgacggggtgaacgtagagcgtgtttttggggctatgctgtgaataaaccacagagcgggacagaacgtggcattcacgccgaaatctttagcattagaaaagtcgaagaatacctgcgcgacaaccccggacaattcacgataaattggtactcatcctggagtccttgtgcagattgcgctgaaaagatcttagaatggtataaccaggagctgcgggggaacggccacactttgaaaatcgaagcttgcaaactctattacgagaaaaatgcgaggaatcaaattgggctgcaaaacctcagagataacggggttgggttgaatgtaggcggaggcggtagcgacgtcggtggaggttcaggagagattcggaagcgaccacttatcgaaacaaacggagaaacaggagaaatcgtgtgggacaagggtagggatttcgcgacagtccggaaggtcctgtccatgccgcaggtgaacatcgttaaaaagaccgaagtacagaccggaggcttctccaaggaaagtatcctcccgaaaaggaacagcgacaagctgatcgcacgcaaaaaagattgggaccccaagaaatacggcggattcgattctcctacagtcgcttacagtgtactggttgtggccaaagtggagaaagggaagtctaaaaaactcaaaagcgtcaaggaactgctgggcatcacaatcatggagcgatcaagcttcgaaaaaaaccccatcgactttctcgaggcgaaaggatataaagaggtcaaaaaagacctcatcattaagcttcccaagtactctctctttgagcttgaaaacggccggaaacgaatgctcgctagtgcgggcgagctgcagaaaggtaacgagctggcactgccctctaaatacgttaatttcttgtatctggccagccactatgaaaagctcaaagggtctcccgaagataatgagcagaagcagctgttcgtggaacaacacaaacactaccttgatgagatcatcgagcaaataagcgaattctccaaaagagtgatcctcgccgacgctaacctcgataaggtgctttctgcttacaataagcacagggataagcccatcagggagcaggcagaaaacattatccacttgtttactctgaccaacttgggcgcgcctgcagccttcaagtacttcgacaccaccatagacagaaagcggtacacctctacaaaggaggtcctggacgccacactgattcatcagtcaattacggggctctatgaaacaagaatcgacctctctcagctcggtggagacagcagggctgaccccaagaagaagaggaaggtgtgatctcttctcgagtcatgtaattagttatgtcacgcttacattcacgccctccccccacatccgctctaaccgaaaaggaaggagttagacaacctgaagtctaggtccctatttatttttttatagttatgttagtattaagaacgttatttatatttcaaatttttcttttttttctgtacagacgcgtgtacgcatgtaacattatactgaaaaccttgcttgagaaggttttgggacgctcgaaggctttaatttgcggccggtacccaattcgccctatagtgagtcgtattacgcgcgctcactggccgtcgttttacaacgtcgtgactgggaaaaccctggcgttacccaacttaatcgccttgcagcacatccccctttcgccagctggcgtaatagcgaagaggcccgcaccgatcgcccttcccaacagttgcgcagcctgaatggcgaatggacgcgccctgtagcggcgcattaagcgcggcgggtgtggtggttacgcgcagcgtgaccgctacacttgccagcgccctagcgcccgctcctttcgctttcttcccttcctttctcgccacgttcgccggctttccccgtcaagctctaaatcgggggctccctttagggttccgatttagtgctttacggcacctcgaccccaaaaaacttgattagggtgatggttcacgtagtgggccatcgccctgatagacggtttttcgccctttgacgttggagtccacgttctttaatagtggactcttgttccaaactggaacaacactcaaccctatctcggtctattcttttgatttataagggattttgccgatttcggcctattggttaaaaaatgagctgatttaacaaaaatttaacgcgaattttaacaaaatattaacgtttacaatttcctgatgcggtattttctccttacgcatctgtgcggtatttcacaccgcatatcgacggtcgaggagaacttctagtatatccacatacctaatattattgccttattaaaaatggaatcccaacaattacatcaaaatccacattctcttcaaaatcaattgtcctgtacttccttgttcatgtgtgttcaaaaacgttatatttataggataattatactctatttctcaacaagtaattggttgtttggccgagcggtctaaggcgcctgattcaagaaatatcttgaccgcagttaactgtgggaatactcaggtatcgtaagatgcaagagttcgaatctcttagcaaccattatttttttcctcaacataacgagaacacacaggggcgctatcgcacagaatcaaattcgatgactggaaattttttgttaatttcagaggtcgcctgacgcatatacctttttcaactgaaaaattgggagaaaaaggaaaggtgagaggccggaaccggcttttcatatagaatagagaagcgttcatgactaaatgcttgcatcacaatacttgaagttgacaatattatttaaggacctattgttttttccaataggtggttagcaatcgtcttactttctaacttttcttaccttttacatttcagcaatatatatatatatttcaaggatataccattctaatgtctgcccctatgtctgcccctaagaagatcgtcgttttgccaggtgaccacgttggtcaagaaatcacagccgaagccattaaggttcttaaagctatttctgatgttcgttccaatgtcaagttcgatttcgaaaatcatttaattggtggtgctgctatcgatgctacaggtgtcccacttccagatgaggcgctggaagcctccaagaaggttgatgccgttttgttaggtgctgtgggtggtcctaaatggggtaccggtagtgttagacctgaacaaggtttactaaaaatccgtaaagaacttcaattgtacgccaacttaagaccatgtaactttgcatccgactctcttttagacttatctccaatcaagccacaatttgctaaaggtactgacttcgttgttgtcagagaattagtgggaggtatttactttggtaagagaaaggaagacgatggtgatggtgtcgcttgggatagtgaacaatacaccgttccagaagtgcaaagaatcacaagaatggccgctttcatggccctacaacatgagccaccattgcctatttggtccttggataaagctaatgttttggcctcttcaagattatggagaaaaactgtggaggaaaccatcaagaacgaattccctacattgaaggttcaacatcaattgattgattctgccgccatgatcctagttaagaacccaacccacctaaatggtattataatcaccagcaacatgtttggtgatatcatctccgatgaagcctccgttatcccaggttccttgggtttgttgccatctgcgtccttggcctctttgccagacaagaacaccgcatttggtttgtacgaaccatgccacggttctgctccagatttgccaaagaataaggtcaaccctatcgccactatcttgtctgctgcaatgatgttgaaattgtcattgaacttgcctgaagaaggtaaggccattgaagatgcagttaaaaaggttttggatgcaggtatcagaactggtgatttaggtggttccaacagtaccaccgaagtcggtgatgctgtcgccgaagaagttaagaaaatccttgcttaaaaagattctctttttttatgatatttgtacataaactttataaatgaaattcataatagaaacgacacgaaattacaaaatggaatatgttcatagggtagacgaaactatatacgcaatctacatacatttatcaagaaggagaaaaaggaggatgtaaaggaatacaggtaagcaaattgatactaatggctcaacgtgataaggaaaaagaattgcactttaacattaatattgacaaggaggagggcaccacacaaaaagttaggtgtaacagaaaatcatgaaactatgattcctaatttatatattggaggattttctctaaaaaaaaaaaaatacaacaaataaaaaacactcaatgacctgaccatttgatggagtttaagtcaataccttcttgaaccatttcccataatggtgaaagttccctcaagaattttactctgtcagaaacggccttacgacgtagtcgatatggtgcactctcagtacaatctgctctgatgccgcatagttaagccagccccgacacccgccaacacccgctgacgcgccctgacgggcttgtctgctcccggcatccgcttacagacaagctgtgaccgtctccgggagctgcatgtgtcagaggttttcaccgtcatcaccgaaacgcgcga

SEQ ID NO: 16 - DNA, 5860 bp, Artificial Sequence
  full-length sequence of vector pAL50
  rep_origin (11)..(599): ori
  gene (773)..(1630): AmpR
  promoter (1631)..(1735): AmpR promoter
  misc_feature (1751)..(1831): Scp1
  misc_feature (1838)..(1847): Kozak sequence
  misc_feature (1844)..(1894): NLS unit
  sig_peptide (1850)..(1870): SV40 NLS
  gene (1895)..(2275): nSaCas9(D10A)
  mutation (1919)..(1921): D10A
  gene (2276)..(2638): HsPmCDA1(30 E150_W122E_W139Q)
  mutation (2552)..(2554): W122E
  misc_feature (2639)..(2671): 6xGS Linker
  gene (2672)..(5446): nSaCas9(D10A)
  sig_peptide (5456)..(5476): SV40 NLS
  gene (5483)..(5734): Ugi
  polyA_signal (5738)..(5786): polyA signal
  promoter (5787)..(5791): H1 promoter
  enhancer (5811)..(5826): CMV enhance
tgctggcgtttttccataggctccgcccccctgacgagcatcacaaaaatcgacgctcaagtcagaggtggcgaaacccgacaggactataaagataccaggcgtttccccctggaagctccctcgtgcgctctcctgttccgaccctgccgcttaccggatacctgtccgcctttctcccttcgggaagcgtggcgctttctcatagctcacgctgtaggtatctcagttcggtgtaggtcgttcgctccaagctgggctgtgtgcacgaaccccccgttcagcccgaccgctgcgccttatccggtaactatcgtcttgagtccaacccggtaagacacgacttatcgccactggcagcagccactggtaacaggattagcagagcgaggtatgtaggcggtgctacagagttcttgaagtggtggcctaactacggctacactagaagaacagtatttggtatctgcgctctgctgaagccagttaccttcggaaaaagagttggtagctcttgatccggcaaacaaaccaccgctggtagcggtggtttttttgtttgcaagcagcagattacgcgcagaaaaaaaggatctcaagaagatcctttgatcttttctacggggtctgacgctcagtggaacgaaaactcacgttaagggattttggtcatgagattatcaaaaaggatcttcacctagatccttttaaattaaaaatgaagttttaaatcaatctaaagtatatatgagtaaacttggtctgacagttaccaatgcttaatcagtgaggcacctatctcagcgatctgtctatttcgttcatccatagttgcctgactccccgtcgtgtagataactacgatacgggagggcttaccatctggccccagtgctgcaatgataccgcgagacccacgctcaccggctccagatttatcagcaataaaccagccagccggaagggccgagcgcagaagtggtcctgcaactttatccgcctccatccagtctattaattgttgccgggaagctagagtaagtagttcgccagttaatagtttgcgcaacgttgttgccattgctacaggcatcgtggtgtcacgctcgtcgtttggtatggcttcattcagctccggttcccaacgatcaaggcgagttacatgatcccccatgttgtgcaaaaaagcggttagctccttcggtcctccgatcgttgtcagaagtaagttggccgcagtgttatcactcatggttatggcagcactgcataattctcttactgtcatgccatccgtaagatgcttttctgtgactggtgagtactcaaccaagtcattctgagaatagtgtatgcggcgaccgagttgctcttgcccggcgtcaatacgggataataccgcgccacatagcagaactttaaaagtgctcatcattggaaaacgttcttcggggcgaaaactctcaaggatcttaccgctgttgagatccagttcgatgtaacccactcgtgcacccaactgatcttcagcatcttttactttcaccagcgtttctgggtgagcaaaaacaggaaggcaaaatgccgcaaaaaagggaataagggcgacacggaaatgttgaatactcatactcttcctttttcaatattattgaagcatttatcagggttattgtctcatgagcggatacatatttgaatgtatttagaaaaataaacaaataggggttccgcggtcgacgtcgctagcgtacttatataagggggtgggggcgcgttcgtcctcagtcgcgatcgaacactcgagccgagcagacgtgcctacggaccgtctagagccaccatggcaccgaagaagaagcgtaaagtcggaatccacggagttcctgcggcaaagcgaaattacattctggggctggccattggcattacatcagtgggctatggcatcattgactacgagacaagggacgtgatcgacgccggcgtgagactgttcaaggaggccaacgtggagaacaatgagggccggagatccaagaggggagcaaggcgcctgaagcggagaaggcgccacagaatccagagagtgaagaagctgctgttcgattacaacctgctgaccgaccactccgagctgtctggcatcaatccttatgaggccagagtgaagggcctgtcccagaagctgtctgaggaggagtttagcgccgccctgctgcacctggcaaagaggagaggcgtgcacaacgtgaatgaggtggaggaggacacctcacaccgctgctacgtgctgtttgagttgaagcgaaggggcgaaagaagggcttgcttttggggctatgccgtcaacaagccccaaagtggcaccgagagaggaatacacgctgagatattcagtatccgaaaggtggaagagtatcttcgggataatcctgggcagtttacgatcaactggtattccagctggagtccttgcgctgattgtgccgagaaaattctggaatggtataatcaggaacttcggggaaacgggcacacattgaaaatcgaagcctgcaagctgtactacgagaagaatgcccggaaccagataggactccagaatctgagggacaatggtgtaggcctgaacgtgggtggaggtggcagtgatgtcggcggaggctccggcaacgagctgtccacaaaggagcagatcagccgcaattccaaggccctggaggagaagtatgtggccgagctgcagctggagcggctgaagaaggatggcgaggtgaggggctccatcaatcgcttcaagacctctgactacgtgaaggaggccaagcagctgctgaaggtgcagaaggcctaccaccagctggatcagtcctttatcgatacatatatcgacctgctggagacaaggcgcacatactatgagggaccaggagagggctctcccttcggctggaaggacatcaaggagtggtacgagatgctgatgggccactgcacctattttccagaggagctgagaagcgtgaagtacgcctataacgccgatctgtacaacgccctgaatgacctgaacaacctggtcatcaccagggatgagaacgagaagctggagtactatgagaagttccagatcatcgagaacgtgttcaagcagaagaagaagcctacactgaagcagatcgccaaggagatcctggtgaacgaggaggacatcaagggctaccgcgtgacctccacaggcaagccagagttcaccaatctgaaggtgtatcacgatatcaaggacatcacagcccggaaggagatcatcgagaacgccgagctgctggatcagatcgccaagatcctgaccatctatcagagctccgaggacatccaggaggagctgaccaacctgaatagcgagctgacacaggaggagatcgagcagatcagcaatctgaagggctacaccggcacacacaacctgagcctgaaggccatcaatctgatcctggatgagctgtggcacacaaacgacaatcagatcgccatctttaaccggctgaagctggtgccaaagaaggtggacctgtcccagcagaaggagatcccaaccacactggtggacgatttcatcctgtctcccgtggtgaagcggagcttcatccagagcatcaaagtgatcaacgccatcatcaagaagtacggcctgcccaatgatatcatcatcgagctggccagggagaagaactccaaggacgcccagaagatgatcaatgagatgcagaagaggaaccgccagaccaatgagcggatcgaggagatcatcagaaccacaggcaaggagaacgccaagtacctgatcgagaagatcaagctgcacgatatgcaggagggcaagtgtctgtattctctggaggccatccctctggaggacctgctgaacaatccattcaactacgaggtggatcacatcatcccccggagcgtgagcttcgacaattcttttaacaataaggtgctggtgaagcaggaggagaacagcaagaagggcaataggacccctttccagtacctgtctagctccgattctaagatcagctacgagacattcaagaagcacatcctgaatctggccaagggcaagggccgcatcagcaagaccaagaaggagtacctgctggaggagcgggacatcaacagattctccgtgcagaaggacttcatcaaccggaatctggtggacaccagatacgccacacgcggcctgatgaatctgctgcggtcttatttcagagtgaacaatctggatgtgaaggtgaagagtatcaacggcggcttcacctcctttctgcggagaaagtggaagtttaagaaggagcgcaacaagggctataagcaccacgccgaggatgccctgatcatcgccaatgccgacttcatctttaaggagtggaagaagctggacaaggccaagaaagtgatggagaaccagatgttcgaggagaagcaggccgagagcatgcccgagatcgagacagagcaggagtacaaggagattttcatcacacctcaccagatcaagcacatcaaggacttcaaggactacaagtattctcacagggtggataagaagcccaaccgcgagctgatcaatgacaccctgtatagcacacggaaggacgataagggcaataccctgatcgtgaacaatctgaacggcctgtacgacaaggataatgacaagctgaagaagctgatcaacaagtctcccgagaagctgctgatgtaccaccacgatcctcagacatatcagaagctgaagctgatcatggagcagtacggcgacgagaagaacccactgtataagtactatgaggagacaggcaactacctgacaaagtatagcaagaaggataatggccccgtgatcaagaagatcaagtactatggcaacaagctgaatgcccacctggacatcaccgacgattaccctaactctcgcaataaggtggtgaagctgagcctgaagccataccggttcgacgtgtacctggacaacggcgtgtataagtttgtgacagtgaagaatctggatgtgatcaagaaggagaactactatgaggtgaacagcaagtgctacgaggaggccaagaagctgaagaagatcagcaaccaggccgagttcatcgcctctttttacaacaatgacctgatcaagatcaatggcgagctgtatagagtgatcggcgtgaacaatgatctgctgaacagaatcgaagtgaatatgatcgacatcacctacagggagtatctggagaacatgaatgataagaggccccctcgcatcatcaagaccatcgcctctaagacacagagcatcaagaagtacagcacagacatcctggggaacctgtatgaagtcaagagcaagaaacatcctcagattatcaagaaaggcggtggaggtcccaagaagaaaagaaaagtcggtaccatgaccaacctttccgacatcatagagaaggaaacaggcaaacagttggtcatccaagagtcgatactcatgcttcctgaagaagttgaggaggtcattgggaataagccggaaagtgacattctcgtacacactgcgtatgatgagagcaccgatgagaacgtgatgctgctcacgtcagatgccccagagtacaaaccctgggctctggtgattcaggactctaatggagagaacaagatcaagatgctatagaataaaagatctttattttcattagatctgtgtgttggttttttgtgtgaattcactagtgggcccacgcgttgacattgattattgaccagcaaaaggccaggaaccgtaaaaaggccgcgt

SEQ ID NO: 17 - DNA, 20 bp, Homo sapiens
gatgttccaatcagtacgca

SEQ ID NO: 18 - DNA, 20 bp, Homo sapiens
gatgttccaatcagtacgca

SEQ ID NO: 19 - DNA, 20 bp, Homo sapiens
gatgttccaatcagtacgca

SEQ ID NO: 20 - DNA, 20 bp, Homo sapiens
gatgttccaatcagtacgca

SEQ ID NO: 21 - protein, 7 aa, Homo sapiens
VRWAKGR

SEQ ID NO: 22 - protein, 22 aa, Homo sapiens
KAWEGLHENSVRLSRQLRRILL

SEQ ID NO: 23 - protein, 7 aa, Petromyzon marinus
QFFNNKK

SEQ ID NO: 24 - protein, 21 aa, Petromyzon marinus
NENRWLEKTLKRAEKRRSELS